European Patent Application EP 4 813 459 A1, published September 30, 2026. Title: ONCOGENIC HCMV-IE1 PROTEIN AND ITS USE IN THE PREVENTION AND TREATMENT OF CANCERS. Applicant: Apex Biosolutions. Application EP. The sequence listing filed with the application follows.

SEQUENCE LISTING (35 sequences)

SEQ ID NO: 1 - DNA, 20 bp, synthetic construct
  source 1..20: mol_type = other DNA
cgacgttcctgcagactatg

SEQ ID NO: 2 - DNA, 20 bp, synthetic construct
  source 1..20: mol_type = other DNA
tcctcggtcacttgttcaaa

SEQ ID NO: 3 - DNA, 20 bp, synthetic construct
  source 1..20: mol_type = other DNA
tcgtgcccttgtgtgatagc

SEQ ID NO: 4 - DNA, 19 bp, synthetic construct
  source 1..19: mol_type = other DNA
tctcggacagccaggtagc

SEQ ID NO: 5 - DNA, 17 bp, synthetic construct
  source 1..17: mol_type = other DNA
acacccttctcccttcg

SEQ ID NO: 6 - DNA, 18 bp, synthetic construct
  source 1..18: mol_type = other DNA
ccgctccacatacagtcc

SEQ ID NO: 7 - DNA, 25 bp, synthetic construct
  source 1..25: mol_type = other DNA
gggaaatggaggggtgcaaaagagg

SEQ ID NO: 8 - DNA, 26 bp, synthetic construct
  source 1..26: mol_type = other DNA
ttgcgtgagtgtggatgggattggtg

SEQ ID NO: 9 - DNA, 23 bp, synthetic construct
  source 1..23: mol_type = other DNA
tcctcctcttcctctatactaac

SEQ ID NO: 10 - DNA, 19 bp, synthetic construct
  source 1..19: mol_type = other DNA
cccacaatcacaggcatag

SEQ ID NO: 11 - DNA, 22 bp, synthetic construct
  source 1..22: mol_type = other DNA
atcccctcaacaacttctcagt

SEQ ID NO: 12 - DNA, 22 bp, synthetic construct
  source 1..22: mol_type = other DNA
cttccgtccactcttctctttc

SEQ ID NO: 13 - DNA, 21 bp, synthetic construct
  source 1..21: mol_type = other DNA
gatgagtatgcctgccgtgtg

SEQ ID NO: 14 - DNA, 19 bp, synthetic construct
  source 1..19: mol_type = other DNA
caatccaaatgcggcatct

SEQ ID NO: 15 - DNA, 45 bp, synthetic construct
  source 1..45: mol_type = other DNA
ctctactagaggatctatttccggtatggagtcctctgccaagag

SEQ ID NO: 16 - DNA, 41 bp, synthetic construct
  source 1..41: mol_type = other DNA
ggagggagaggggcgggatcctattactggtcagccttgct

SEQ ID NO: 17 - DNA, 18 bp, synthetic construct
  source 1..18: mol_type = other DNA
gcattcctttggcgagag

SEQ ID NO: 18 - DNA, 21 bp, synthetic construct
  source 1..21: mol_type = other DNA
cgcaaatgggcggtaggcgtg

SEQ ID NO: 19 - DNA, 20 bp, synthetic construct
  source 1..20: mol_type = other DNA
ccaatggctgcagtcaggcc

SEQ ID NO: 20-21 - skipped (2 entries)

SEQ ID NO: 22 - protein, 5 aa, synthetic construct
LKTFE

SEQ ID NO: 23 - protein, 10 aa, synthetic construct
EESLKTFEQV

SEQ ID NO: 24 - protein, 23 aa, synthetic construct
EESLKTFEQVTEDCNENPELDVL

SEQ ID NO: 25 - protein, 491 aa, synthetic construct
MESSAKRKMDPDNPDEGPSSKVPRPETPVTKATTFLQTMLRKEVNSQLSLGDPLFPELAEESLKTFEQVTEDCNENPEKDVLTELVKQIKVRVDMVRHRIKEHMLKKYTQTEEKFTGAFNMMGGCLQNALDILDKVHEPFEEMKCIGLTMQSMYENYIVPEDKREMWMACIKELHDVSKGAANKLGGALQAKARAKKDELRRKMMYMCYRNIEFFTKNSAFPKTTNGCSQAMAALQNLPQCSPDEIMAYAQKIFKILDEERDKVLTHIDHIFMDILTTCVETMCNEYKVTSDACMMTMYGGISLLSEFCRVLCCYVLEETSVMLAKRPLITKPEVISVMKRRIEEICMKVFAQYILGADPLRVCSPSVDDLRAIAEESDEEEAIAAYTLATAGASSSDSLVSPPESPVPATIPLSSVIVAENSDQEESEQSDEEQEEGAQEEREDTVSVKSEPVSEIGEVAPEEEEDGAEEPTTSGGKSTHPMVTRSKADQ

SEQ ID NO: 26 - DNA, 15 bp, synthetic construct
  source 1..15: mol_type = other DNA
ttcaaaagttttgag

SEQ ID NO: 27 - DNA, 20 bp, synthetic construct
  source 1..20: mol_type = other DNA
cgacgttcctgcagactatg

SEQ ID NO: 28 - DNA, 20 bp, synthetic construct
  source 1..20: mol_type = other DNA
tcctcggtcacttgttcaaa

SEQ ID NO: 29 - DNA, 25 bp, synthetic construct
  source 1..25: mol_type = other DNA
cagggacagcagagatccagtttat

SEQ ID NO: 30 - DNA, 33 bp, synthetic construct
  source 1..33: mol_type = other DNA
ctcggtcacttgtgaagcagttttgagggattc

SEQ ID NO: 31 - DNA, 33 bp, synthetic construct
  source 1..33: mol_type = other DNA
gaatccctcaaaactgcttcacaagtgaccgag

SEQ ID NO: 32 - DNA, 18 bp, synthetic construct
  source 1..18: mol_type = other DNA
gcattcctttggcgagag

SEQ ID NO: 33 - DNA, 21 bp, synthetic construct
  source 1..21: mol_type = other DNA
cgcaaatgggcggtaggcgtg

SEQ ID NO: 34 - DNA, 20 bp, synthetic construct
  source 1..20: mol_type = other DNA
ccaatggctgcagtcaggcc

SEQ ID NO: 35 - DNA, 15 bp, synthetic construct
  source 1..15: mol_type = other DNA
ctcaaaacttttgaa